European Patent Application EP 4 461 814 A2, published November 13, 2024. Title: GENERATION OF IMPROVED HUMAN PAH FOR TREATMENT OF SEVERE PKU BY LIVER-DIRECTED GENE REPLACEMENT THERAPY. Applicant: GENZYME CORPORATION. Application EP. The sequence listing filed with the application follows.

SEQUENCE LISTING (18 sequences)

SEQ ID NO: 1 - protein, 452 aa, Homo sapiens
MSTAVLENPGLGRKLSDFGQETSYIEDNCNQNGAISLIFSLKEEVGALAKVLRLFEENDVNLTHIESRPSRLKKDEYEFFTHLDKRSLPALTNIIKILRHDIGATVHELSRDKKKDTVPWFPRTIQELDRFANQILSYGAELDADHPGFKDPVYRARRKQFADIAYNYRHGQPIPRVEYMEEEKKTWGTVFKTLKSLYKTHACYEYNHIFPLLEKYCGFHEDNIPQLEDVSQFLQTCTGFRLRPVAGLLSSRDFLGGLAFRVFHCTQYIRHGSKPMYTPEPDICHELLGHVPLFSDRSFAQFSQEIGLASLGAPDEYIEKLATIYWFTVEFGLCKQGDSIKAYGAGLLSSFGELQYCLSEKPKLLPLELEKTAIQNYTVTEFQPLYYVAESFNDAKEKVRNFAATIPRPFSVRYDPYTQRIEVLDNTQQLKILADSINSEIGILCSALQKIK

SEQ ID NO: 2 - protein, 452 aa, Homo sapiens
MSTAVLENPGLGRKLSDFGQETSYIEDNCNQNGAISLIFSLKEEVGALAKVLRLFEENDVNLTHIESRPSRLKKDEYEFFTHLDKRSLPALTNIIKILRHDIGATVHELSRDKKKDTVPWFPRTIQELDRFANQILSYGAELDADHPGFKDPVYRARRKQFADIAYNYRHGQPIPRVEYMEEGKKTWGTVFKTLKSLYKTHACYEYNHIFPLLEKYCGFHEDNIPQLEDVSQFLQTCTGFRLRPVAGLLSSRDFLGGLAFRVFHCTQYIRHGSKPMYTPEPDICHELLGHVPLFSDRSFAQFSQEIGLASLGAPDEYIEKLATIYWFTVEFGLCKQGDSIKAYGAGLLSSFGELQYCLSEKPKLLPLELEKTAIQNYTVTEFQPLYYVAESFNDAKEKVRNFAATIPRPFSVRYDPYTQRIEVLDNTQQLKILADSINSEIGILCSALQKIK

SEQ ID NO: 3 - protein, 452 aa, Homo sapiens
MSTAVLENPGLGRKLSDFGQETSYIEDNCNQNGAISLIFSLKEEVGALAKVLRLFEENDVNLTHIESRPSRLKKDEYEFFTHLDKRSLPALTNIIKILRHDIGATVHELSRDKKKDTVPWFPRTIQELDRFANQILSYGAELDADHPGFKDPVYRARRKQFADIAYNYRHGQPIPRVEYTEEEKKTWGTVFKTLKSLYPTHACYEYNHIFPLLEKYCGFHEDNIPQLEDVSQFLQTCTGFRLRPVAGLLPSRDFLAGLAFRVFHCTQYIRHGSKPMYTPEPDICHELLGHVPLFSDRSFAQFSQEIGLASLGAPDEYIEKLATIYWFTVEFGLCKQGDSIKAYGAGLLSSFGELQYCLSEKPKLLPLELEKTAIQNYTVTEFQPLYYVAESFNDAKEKVRNFAATIPRPFSVRYDPYTQRIEVLDNTQQLKILADSINSEIGILCSALQKIK

SEQ ID NO: 4 - DNA, 1359 bp, Homo sapiens
  source 1..1359: mol_type = other DNA
atgagcacagccgtgctggaaaaccccggcctgggcagaaagctgagcgacttcggccaggaaaccagctacatcgaggacaactgcaaccagaacggcgccatcagcctgatcttcagcctgaaagaagaagtgggcgccctggccaaggtgctgcggctgttcgaggagaacgacgtgaacctgacccacatcgagagccggcccagcagactgaagaaggacgagtacgagttcttcacccacctggacaagcggagcctgcccgccctgaccaacatcatcaagatcctgcggcacgacatcggcgccaccgtgcacgagctgagccgggacaagaaaaaggacaccgtgccctggttccccagaaccatccaggaactggacagattcgccaaccagatcctgtcctacggcgccgagctggatgccgaccaccctggcttcaaggaccccgtgtaccgggccagacggaagcagttcgccgatatcgcctacaactaccggcacggccagcccatccccagagtcgagtacaccgaagagggcaagaaaacctggggcaccgtgttcaagaccctgaagtccctgtaccccacccacgcctgctacgagtacaaccacatcttcccactgctcgaaaagtactgcggcttccacgaggacaatatccctcagctggaggacgtgtcccagtttctgcagacctgcaccggcttcagactcaggcctgtggccggcctgctgcccagcagagattttctggccggactggccttccgggtgttccactgcacccagtacatcagacacggcagcaagcccatgtacacccctgagcccgacatctgccacgagctgctgggacatgtgcccctgttcagcgacagaagcttcgcccagttcagccaggaaatcggcctggcctctctgggcgctcccgacgagtatatcgagaagctggccaccatctactggttcaccgtggaattcggcctgtgcaagcagggcgacagcatcaaggcctatggcgccggactcctgtccagcttcggcgagctgcagtactgtctgagcgagaagcccaagctgctgcccctggaactggaaaagaccgccatccagaactacaccgtgaccgagttccagcccctgtactacgtggccgagagcttcaacgacgccaaagaaaaagtgcggaacttcgccgccaccatccctcggcccttcagcgtcagatacgacccctacacccagcggatcgaggtgctggacaacacacagcagctgaaaattctggccgactccatcaacagcgagatcggcatcctgtgcagcgccctgcagaaaatcaagtga

SEQ ID NO: 5 - DNA, 3713 bp, synthetic construct
  misc_feature 1..3713: note = Synthetic Construct
  source 1..3713: mol_type = other DNA
gagctcttggccactccctctctgcgcgctcgctcgctcactgaggccgggcgaccaaaggtcgcccgacgcccgggctttgcccgggcggcctcagtgagcgagcgagcgcgcagagagggagtggccaactccatcactaggggttcctacgcgtggccccaggttaatttttaaaaagcagtcaaaggtcaaagtggcccttggcagcatttactctctctattgactttggttaataatctcaggagcacaaacattcctggaggcaggagaagaaatcaacatcctggacttatcctctgggcctctccccaccttcgatggccccaggttaatttttaaaaagcagtcaaaggtcaaagtggcccttggcagcatttactctctctattgactttggttaataatctcaggagcacaaacattcctggaggcaggagaagaaatcaacatcctggacttatcctctgggcctctccccaccgatatctacctgctgatcgcccggcccctgttcaaacatgtcctaatactctgtcggggcaaaggtcggcagtagttttccatcttactcaacatcctcccagtgtacgtaggatcctgtctgtctgcacatttcgtagagcgagtgttccgatactctaatctcccggggcaaaggtcgtattgacttaggttacttattctccttttgttgactaagtcaataatcagaatcagcaggtttggagtcagcttggcagggatcagcagcctgggttggaaggagggggtataaaagccccttcaccaggagaagccgtcacacagatccacaagctcctgctagcagtcgctgcgcgctgccttcgccccgtgccccgctccgccgccgcctcgcgccgcccgccccggctctgactgaccgcgttactcccacaggtgagcgggcgggacggcccttctcctccgggctgtaattagcgcttggtttaatgacggcttgtttcttttctgtggctgcgtgaaagccttgaggggctccgggaaggccctttgtgcggggggagcggctcggggggtgcgtgcgtgtgtgtgtgcgtggggagcgccgcgtgcggctccgcgctgcccggcggctgtgagcgctgcgggcgcggcgcggggctttgtgcgctccgcagtgtgcgcgaggggagcggggccgggggcggtgccccgcggtgcggggggggctgcgaggggaacaaaggctgcgtgcggggtgtgtgcgtgggggggtgagcagggggtgtgggcgcgtcggtcgggctgcaaccccccctgcacccccctccccgagttgctgagcacggcccggcttcgggtgcggggctccgtacggggcgtggcgcggggctcgccgtgccgggcggggggtggcggcaggtgggggtgccgggcggggcggggccgcctcgggccggggagggctcgggggaggggcgcggcggcccccggagcgccggcggctgtcgaggcgcggcgagccgcagccattgccttttatggtaatcgtgcgagagggcgcagggacttcctttgtcccaaatctgtgcggagccgaaatctgggaggcgccgccgcaccccctctagcgggcgcggggcgaagcggtgcggcgccggcaggaaggaaatgggcggggagggccttcgtgcgtcgccgcgccgccgtccccttctccctctccagcctcggggctgtccgcggggggacggctgccttcgggggggacggggcagggcggggttcggcttctggcgtgtgaccggcggctctagagcctctgctaaccatgttcatgccttcttctttttcctacagctcctgggcaacgtgctggttattgtgctgtctcatcattttggcaaagaattcatttcgaagccgccaccatgagcacagccgtgctggaaaaccccggcctgggcagaaagctgagcgacttcggccaggaaaccagctacatcgaggacaactgcaaccagaacggcgccatcagcctgatcttcagcctgaaagaagaagtgggcgccctggccaaggtgctgcggctgttcgaggagaacgacgtgaacctgacccacatcgagagccggcccagcagactgaagaaggacgagtacgagttcttcacccacctggacaagcggagcctgcccgccctgaccaacatcatcaagatcctgcggcacgacatcggcgccaccgtgcacgagctgagccgggacaagaaaaaggacaccgtgccctggttccccagaaccatccaggaactggacagattcgccaaccagatcctgtcctacggcgccgagctggatgccgaccaccctggcttcaaggaccccgtgtaccgggccagacggaagcagttcgccgatatcgcctacaactaccggcacggccagcccatccccagagtcgagtacaccgaagagggcaagaaaacctggggcaccgtgttcaagaccctgaagtccctgtaccccacccacgcctgctacgagtacaaccacatcttcccactgctcgaaaagtactgcggcttccacgaggacaatatccctcagctggaggacgtgtcccagtttctgcagacctgcaccggcttcagactcaggcctgtggccggcctgctgcccagcagagattttctggccggactggccttccgggtgttccactgcacccagtacatcagacacggcagcaagcccatgtacacccctgagcccgacatctgccacgagctgctgggacatgtgcccctgttcagcgacagaagcttcgcccagttcagccaggaaatcggcctggcctctctgggcgctcccgacgagtatatcgagaagctggccaccatctactggttcaccgtggaattcggcctgtgcaagcagggcgacagcatcaaggcctatggcgccggactcctgtccagcttcggcgagctgcagtactgtctgagcgagaagcccaagctgctgcccctggaactggaaaagaccgccatccagaactacaccgtgaccgagttccagcccctgtactacgtggccgagagcttcaacgacgccaaagaaaaagtgcggaacttcgccgccaccatccctcggcccttcagcgtcagatacgacccctacacccagcggatcgaggtgctggacaacacacagcagctgaaaattctggccgactccatcaacagcgagatcggcatcctgtgcagcgccctgcagaaaatcaagtgacctaggtgatcaagatctgctagcttaattaacccgggactagtgcggccgctcgagactagtctgtgccttctagttgccagccatctgttgtttgcccctcccccgtgccttccttgaccctggaaggtgccactcccactgtcctttcctaataaaatgaggaaattgcatcgcattgtctgagtaggtgtcattctattctggggggtggggtggggcaggacagcaagggggaggattgggaagacaatagcaggcatgctggggatgcggtgggctctatggtaccaggaacccctagtgatggagttggccactccctctctgcgcgctcgctcgctcactgaggccgggcgaccaaaggtcgcccgacgcccgggctttgcccgggcggcctcagtgagcgagcgagcgcgcagagagggagtggcc

SEQ ID NO: 6 - DNA, 4561 bp, synthetic construct
  misc_feature 1..4561: note = Synthetic Construct
  source 1..4561: mol_type = other DNA
ttggccactccctctctgcgcgctcgctcgctcactgaggccgcccgggcaaagcccgggcgtcgggcgacctttggtcgcccggcctcagtgagcgagcgagcgcgcagagagggagtggccaactccatcactaggggttccttaccgcgtggccccaggttaatttttaaaaagcagtcaaaggtcaaagtggcccttggcagcatttactctctctattgactttggttaataatctcaggagcacaaacattcctggaggcaggagaagaaatcaacatcctggacttatcctctgggcctctccccaccttcgatggccccaggttaatttttaaaaagcagtcaaaggtcaaagtggcccttggcagcatttactctctctattgactttggttaataatctcaggagcacaaacattcctggaggcaggagaagaaatcaacatcctggacttatcctctgggcctctccccaccgatatctacctgctgatcgcccggcccctgttcaaacatgtcctaatactctgtcggggcaaaggtcggcagtagttttccatcttactcaacatcctcccagtgtacgtaggatcctgtctgtctgcacatttcgtagagcgagtgttccgatactctaatctcccggggcaaaggtcgtattgacttaggttacttattctccttttgttgactaagtcaataatcagaatcagcaggtttggagtcagcttggcagggatcagcagcctgggttggaaggagggggtataaaagccccttcaccaggagaagccgtcacacagatccacaagctcctgctagccaattgagtcgctgcgcgctgccttcgccccgtgccccgctccgccgccgcctcgcgccgcccgccccggctctgactgaccgcgttactcccacaggtgagcgggcgggacggcccttctcctccgggctgtaattagcgcttggtttattgacggcttgtttcttttctgtggctgcgtgaaagccttgaggggctccgggaaggccctttgtgcggggggagcggctcggggggtgcgtgcgtgtgtgtgtgcgtggggagcgccgcgtgcggctccgcgctgcccggcggctgtgagcgctgcgggcgcggcgcggggctttgtgcgctccgcagtgtgcgcgaggggagcggggccgggggcggtgccccgcggtgcggggggggctgcgaggggaacaaaggctgcgtgcggggtgtgtgcgtgggggggtgagcagggggtgtgggcgcgtcggtcgggctgcaaccccccctgcacccccctccccgagttgctgagcacggcccggcttcgggtgcggggctccgtacggggcgtggcgcggggctcgccgtgccgggcggggggtggcggcaggtgggggtgccgggcggggcggggccgcctcgggccggggagggctcgggggaggggcgcggcggcccccggagcgccggcggctgtcgaggcgcggcgagccgcagccattgccttttttggtaatcgtgcgagagggcgcagggacttcctttgtcccaaatctgtgcggagccgaaatctgggaggcgccgccgcaccccctctagcgggcgcggggcgaagcggtgcggcgccggcaggaaggaattgggcggggagggccttcgtgcgtcgccgcgccgccgtccccttctccctctccagcctcggggctgtccgcggggggacggctgccttcgggggggacggggcagggcggggttcggcttctggcgtgtgaccggcggctctagagcctctgctaaccttgttcttgccttcttctttttcctacagctcctgggcaacgtgctggttattgtgctgtctcatcattttggcaaagaattcatttcgaagccgccaccatgagcacagccgtgctggaaaaccccggcctgggcagaaagctgagcgacttcggccaggaaaccagctacatcgaggacaactgcaaccagaacggcgccatcagcctgatcttcagcctgaaagaagaagtgggcgccctggccaaggtgctgcggctgttcgaggagaacgacgtgaacctgacccacatcgagagccggcccagcagactgaagaaggacgagtacgagttcttcacccacctggacaagcggagcctgcccgccctgaccaacatcatcaagatcctgcggcacgacatcggcgccaccgtgcacgagctgagccgggacaagaaaaaggacaccgtgccctggttccccagaaccatccaggaactggacagattcgccaaccagatcctgtcctacggcgccgagctggatgccgaccaccctggcttcaaggaccccgtgtaccgggccagacggaagcagttcgccgatatcgcctacaactaccggcacggccagcccatccccagagtcgagtacaccgaagagggcaagaaaacctggggcaccgtgttcaagaccctgaagtccctgtaccccacccacgcctgctacgagtacaaccacatcttcccactgctcgaaaagtactgcggcttccacgaggacaatatccctcagctggaggacgtgtcccagtttctgcagacctgcaccggcttcagactcaggcctgtggccggcctgctgcccagcagagattttctggccggactggccttccgggtgttccactgcacccagtacatcagacacggcagcaagcccatgtacacccctgagcccgacatctgccacgagctgctgggacatgtgcccctgttcagcgacagaagcttcgcccagttcagccaggaaatcggcctggcctctctgggcgctcccgacgagtatatcgagaagctggccaccatctactggttcaccgtggaattcggcctgtgcaagcagggcgacagcatcaaggcctatggcgccggactcctgtccagcttcggcgagctgcagtactgtctgagcgagaagcccaagctgctgcccctggaactggaaaagaccgccatccagaactacaccgtgaccgagttccagcccctgtactacgtggccgagagcttcaacgacgccaaagaaaaagtgcggaacttcgccgccaccatccctcggcccttcagcgtcagatacgacccctacacccagcggatcgaggtgctggacaacacacagcagctgaaaattctggccgactccatcaacagcgagatcggcatcctgtgcagcgccctgcagaaaatcaagtgaactagtctgtgccttctagttgccagccatctgttgtttgcccctcccccgtgccttccttgaccctggaaggtgccactcccactgtcctttcctaataaaatgaggaaattgcatcgcattgtctgagtaggtgtcattctattctggggggtggggtggggcaggacagcaagggggaggattgggaagacaatagcaggcatgctggggatgcggtgggctctataccggtccaggggtgagtgaaggtttggaagagtgtagcagaataagaaaccatgagtcccctccctgagaagccctgagcccccttgacgacacacatccctcgaggctcagcttcatcatctgtaaaaggtgctgaaactgaccatccaagctgccgaaaaagattgtgtggggataattcaaaactagaggaagatgcagaatttctacatcgtggcgatgtcaggctaagagttgccatcgtggctgtccatcgattttattggaatcatatgtttatttgagggtgtcttggatattacaaataaattgttggagcatcaggcatatttggtaattctgtctaaggctccctgccccttgttaattggcagctcagttattcatccagggcaaacattctgcttactattcctgagagctttcctcatcctctagattggcaggggaattgcagttgcctgagcagcctcccctctgccataccaacagagcttcaccatcgaggcttgcagagtggacaggggcctcagggacccctgatcccagctttctcattggacagaaggaggagactggggctggagagggacctgggcccccactaaggccacagcagagccaggactttagctgtgctgactgcagcctggcttgcctccactgccctcctttgcctcaagagcaagggagcctcagagtggaggaagcagcccctggccttgcctcccacctcccctcccctttgctgttttcctgggacagtgggagctggcttagattgccctggggcccccaggaccctggcattttaacccctcaggggcaggaaggcagcctgagatacagaagagtccatcacctgctgtatgccacacaccatccccacagtcgacatttaaattaggaacccctagtgatggagttggccactccctctctgcgcgctcgctcgctcactgaggccgcccgggcaaagcccgggcgtcgggcgacctttggtcgcccggcctcagtgagcgagcgagcgcgcagagagggagtggccaa

SEQ ID NO: 7 - DNA, 204 bp, synthetic construct
  misc_feature 1..204: note = Synthetic Construct
  source 1..204: mol_type = other DNA
gcgagaacttgtgcctccccgtgttcctgacctttgaccctctgtcctacttagactaatattgactttgggtactgcaaacaggaaatgggggagggattcgatgcgagaacttgtgcctccccgtgttcctgacctttgaccctctgtcctacttagactaatattgactttgggtactgcaaacaggaaatgggggaggga

SEQ ID NO: 8 - DNA, 330 bp, synthetic construct
  misc_feature 1..330: note = Synthetic Construct
  source 1..330: mol_type = other DNA
ggccccaggttaatttttaaaaagcagtcaaaggtcaaagtggcccttggcagcatttactctctctattgactttggttaataatctcaggagcacaaacattcctggaggcaggagaagaaatcaacatcctggacttatcctctgggcctctccccaccttcgatggccccaggttaatttttaaaaagcagtcaaaggtcaaagtggcccttggcagcatttactctctctattgactttggttaataatctcaggagcacaaacattcctggaggcaggagaagaaatcaacatcctggacttatcctctgggcctctccccacc

SEQ ID NO: 9 - DNA, 377 bp, synthetic construct
  misc_feature 1..377: note = Synthetic Construct
  source 1..377: mol_type = other DNA
gttcctagattacattacacattctgcaagcatagcacaggtcaaagttcaactttaattactttcattttcttgtatcctcacagcctagaaaataacctgcgttacagcatccactcagtatcccttgagcatgaggtgacactacttaacatagggacgagatggtactttgtgtctcctgctctgtcagcagggcactgtacttgctgataccagggaatattgatttgtaaataccatcattccgaacgtgtttgccttggccagttttccatgtacatgcagaaagaagtttgggactgatcaatacagtcctctgcctttaaagcaataggaaaaggccaacttgtctacgtttagtatgtggctgtaga

SEQ ID NO: 10 - DNA, 156 bp, synthetic construct
  misc_feature 1..156: note = Synthetic Construct
  source 1..156: mol_type = other DNA
ccatcagatcctgcccaaggtcttacataagaggactcttggactcccagcaatgtcaacgaccgaccttgaggcctacttcaaagactgtgtgtttaaggactgggaggagctgggggaggagattaggttaaaggtctttgtattaggaggctg

SEQ ID NO: 11 - DNA, 71 bp, synthetic construct
  misc_feature 1..71: note = Synthetic Construct
  source 1..71: mol_type = other DNA
ggggaggctgctggtgaatattaaccaaggtcaccccagttatcggaggagcaaacaggggctaagtccac

SEQ ID NO: 12 - DNA, 869 bp, synthetic construct
  misc_feature 1..869: note = Synthetic Construct
  source 1..869: mol_type = other DNA
ctcaattggatgacactagtcatcacatttaaaagcatctcaggtaactatattttgaattttttaaaaaagtaactataatagttattattaaaatagcaaagattgaccatttccaagagccatatagaccagcaccgaccactattctaaactatttatgtatgtaaatattagcttttaaaattctcaaaatagttgctgagttgggaaccactattatttctatcgattcagcagccgtaagtctaggacaggcttaaattgttttcactggtgtaaattgcagaaagatgatctaagtaatttggcatttattttaataggtttgaaaaacacatgccattttacaaataagacttatatttgtccttttgtttttcagcctaccatgagaataagagaaagaaaatgaagatcaaaagcttattcatctgtttttctttttcgttggtgtaaagccaacaccctgtctaaaaaacataaatttctttaatcattttgcctcttttctctgtgcttcaattaataaaaaatggaaagaatctaatagagtggtacagcactgttatttttcaaagatgtgttgctatcctgaaaattctgtaggttctgtggaagttccagtgttctctcttattccacttcggtagaggatttctagtttcttgtgggctaattaaataaatcattaatactcttctaagttatggattataaacattcaaaataatattttgacattatgataattctgaataaaagaacaaaaaccatggtataggtaaggaatataaaacatggcttttaccttagaaaaaacaattctaaaattcatatggaatcaaaaaagagcctgcaggtaccct

SEQ ID NO: 13 - DNA, 1302 bp, synthetic construct
  misc_feature 1..1302: note = Synthetic Construct
  source 1..1302: mol_type = other DNA
ctcaattggatgacactagtcatcacatttaaaagcatctcaggtaactatattttgaattttttaaaaaagtaactataatagttattattaaaatagcaaagattgaccatttccaagagccatatagaccagcaccgaccactattctaaactatttatgtatgtaaatattagcttttaaaattctcaaaatagttgctgagttgggaaccactattatttctatctactgttttaattaaaattatctctaaggcatgtgaactggctgtcttggttttcatctgtacttcatctgctacctctgtgacctgaaacatatttataattccattaagctgtgcatatgatagatttatcatatgtattttccttaaaggatttttgtaagaactaattgaattgatacctgtaaagtctttatcacactacccaataaataataaatctctttgttcagctctctgtttctataaatatgtaccagttttattgtttttagtggtagtgattttattctctttctatatatatacacacacatgtgtgcattcataaatatatacaatttttatgaataaaaaattattagcaatcaatattgaaaaccactgatttttgtttatgtgagcaaacagcagattaaaaggaattcctgcagattcagcagccgtaagtctaggacaggcttaaattgttttcactggtgtaaattgcagaaagatgatctaagtaatttggcatttattttaataggtttgaaaaacacatgccattttacaaataagacttatatttgtccttttgtttttcagcctaccatgagaataagagaaagaaaatgaagatcaaaagcttattcatctgtttttctttttcgttggtgtaaagccaacaccctgtctaaaaaacataaatttctttaatcattttgcctcttttctctgtgcttcaattaataaaaaatggaaagaatctaatagagtggtacagcactgttatttttcaaagatgtgttgctatcctgaaaattctgtaggttctgtggaagttccagtgttctctcttattccacttcggtagaggatttctagtttcttgtgggctaattaaataaatcattaatactcttctaagttatggattataaacattcaaaataatattttgacattatgataattctgaataaaagaacaaaaaccatggtataggtaaggaatataaaacatggcttttaccttagaaaaaacaattctaaaattcatatggaatcaaaaaagagcctgcaggtaccct

SEQ ID NO: 14 - DNA, 1359 bp, synthetic construct
  misc_feature 1..1359: note = Synthetic Construct
  source 1..1359: mol_type = other DNA
atgagcacagccgtgctggaaaaccccggcctgggcagaaagctgagcgacttcggccaggaaaccagctacatcgaggacaactgcaaccagaacggcgccatcagcctgatcttcagcctgaaagaagaagtgggcgccctggccaaggtgctgcggctgttcgaagagaacgacgtgaacctgacccacatcgagagccggcccagcagactgaagaaggacgagtacgagttcttcacccacctggacaagcggagcctgcccgccctgaccaacatcatcaagatcctgcggcacgacatcggcgccaccgtgcacgagctgagccgggacaagaaaaaggacaccgtgccctggttccccagaaccatccaggaactggacagattcgccaaccagatcctgtcctacggcgccgagctggatgccgaccaccctggcttcaaggaccccgtgtaccgggccagacggaagcagttcgccgatatcgcctacaactaccggcacggccagcccatccccagagtcgagtacatggaagagggcaagaaaacctggggcaccgtgttcaagaccctgaagtccctgtacaagacccacgcctgctacgagtacaaccacatcttcccactgctcgagaagtactgcggcttccacgaggacaatatccctcagctcgaggacgtgtcccagtttctgcagacctgcaccggcttcagactcaggcctgtggccggcctgctgagcagcagagattttctgggcggactggccttccgggtgttccactgcacccagtacatcagacacggcagcaagcccatgtacacccctgagcccgacatctgccacgagctgctgggacatgtgcccctgttcagcgacagaagcttcgcccagttcagccaggaaatcggcctggcctctctgggcgctcccgacgagtatatcgagaagctggccaccatctactggttcaccgtggaattcggcctgtgcaagcagggcgacagcatcaaggcctatggcgccggactcctgtccagcttcggcgagctgcagtactgtctgagcgagaagcccaagctgctgcccctggaactggaaaagaccgccatccagaactacaccgtgaccgagttccagcccctgtactacgtggccgagagcttcaacgacgccaaagaaaaagtgcggaacttcgccgccaccatccctcggcccttcagcgtcagatacgacccctacacccagcggatcgaggtgctggacaacacacagcagctgaaaattctggccgactccatcaacagcgagatcggcatcctgtgcagcgccctgcagaaaatcaagtga

SEQ ID NO: 15 - DNA, 1069 bp, synthetic construct
  misc_feature 1..1069: note = Synthetic Construct
  source 1..1069: mol_type = other DNA
agtcgctgcgcgctgccttcgccccgtgccccgctccgccgccgcctcgcgccgcccgccccggctctgactgaccgcgttactcccacaggtgagcgggcgggacggcccttctcctccgggctgtaattagcgcttggtttattgacggcttgtttcttttctgtggctgcgtgaaagccttgaggggctccgggaaggccctttgtgcggggggagcggctcggggggtgcgtgcgtgtgtgtgtgcgtggggagcgccgcgtgcggctccgcgctgcccggcggctgtgagcgctgcgggcgcggcgcggggctttgtgcgctccgcagtgtgcgcgaggggagcggggccgggggcggtgccccgcggtgcggggggggctgcgaggggaacaaaggctgcgtgcggggtgtgtgcgtgggggggtgagcagggggtgtgggcgcgtcggtcgggctgcaaccccccctgcacccccctccccgagttgctgagcacggcccggcttcgggtgcggggctccgtacggggcgtggcgcggggctcgccgtgccgggcggggggtggcggcaggtgggggtgccgggcggggcggggccgcctcgggccggggagggctcgggggaggggcgcggcggcccccggagcgccggcggctgtcgaggcgcggcgagccgcagccattgccttttttggtaatcgtgcgagagggcgcagggacttcctttgtcccaaatctgtgcggagccgaaatctgggaggcgccgccgcaccccctctagcgggcgcggggcgaagcggtgcggcgccggcaggaaggaattgggcggggagggccttcgtgcgtcgccgcgccgccgtccccttctccctctccagcctcggggctgtccgcggggggacggctgccttcgggggggacggggcagggcggggttcggcttctggcgtgtgaccggcggctctagagcctctgctaaccttgttcttgccttcttctttttcctacagctcctgggcaacgtgctggttattgtgctgtctcatcattttggcaaagaattc

SEQ ID NO: 16 - DNA, 901 bp, synthetic construct
  misc_feature 1..901: note = Synthetic Construct
  source 1..901: mol_type = other DNA
ccaggggtgagtgaaggtttggaagagtgtagcagaataagaaaccatgagtcccctccctgagaagccctgagcccccttgacgacacacatccctcgaggctcagcttcatcatctgtaaaaggtgctgaaactgaccatccaagctgccgaaaaagattgtgtggggataattcaaaactagaggaagatgcagaatttctacatcgtggcgatgtcaggctaagagttgccatcgtggctgtccatcgattttattggaatcatatgtttatttgagggtgtcttggatattacaaataaattgttggagcatcaggcatatttggtaattctgtctaaggctccctgccccttgttaattggcagctcagttattcatccagggcaaacattctgcttactattcctgagagctttcctcatcctctagattggcaggggaattgcagttgcctgagcagcctcccctctgccataccaacagagcttcaccatcgaggcttgcagagtggacaggggcctcagggacccctgatcccagctttctcattggacagaaggaggagactggggctggagagggacctgggcccccactaaggccacagcagagccaggactttagctgtgctgactgcagcctggcttgcctccactgccctcctttgcctcaagagcaagggagcctcagagtggaggaagcagcccctggccttgcctcccacctcccctcccctttgctgttttcctgggacagtgggagctggcttagattgccctggggcccccaggaccctggcattttaacccctcaggggcaggaaggcagcctgagatacagaagagtccatcacctgctgtatgccacacaccatccccacagtcgacatttaaatt

SEQ ID NO: 17 - DNA, 78 bp, synthetic construct
  misc_feature 1..78: note = Synthetic Construct
  source 1..78: mol_type = other DNA
cactccctctctgcgcgctcgctcgctcactgaggccgggcgaccaaaggtcgcccacgcccgggctttgcccgggcg

SEQ ID NO: 18 - protein, 23 aa, synthetic construct
  REGION 1..23: note = Synthetic Construct
MDYKDHDGDYKDHDIDYKDDDDK